European Patent Application EP 4 293 045 A1, published December 20, 2023. Title: ANTI-TIGIT ANTIBODY PHARMACEUTICAL COMPOSITION AND APPLICATION THEREOF. Applicant: SHANGHAI JUNSHI BIOSCIENCES CO., LTD. SUZHOU JUNMENG BIOSCIENCES CO., LTD. The sequence listing filed with the application follows.

SEQUENCE LISTING (14 sequences)

SEQ ID NO: 1 - protein, 8 aa, Artificial Sequence
  HCDR1
GYAFTEYT

SEQ ID NO: 2 - protein, 8 aa, Artificial Sequence
  HCDR2
INPNTGGT

SEQ ID NO: 3 - protein, 12 aa, Artificial Sequence
  HCDR3
AKLLRLMYYFDY

SEQ ID NO: 4 - protein, 6 aa, Artificial Sequence
  LCDR1
QDVRTA

SEQ ID NO: 5 - protein, 3 aa, Artificial Sequence
  LCDR2
SAS

SEQ ID NO: 6 - protein, 9 aa, Artificial Sequence
  LCDR3
HQHYITPWT

SEQ ID NO: 7 - protein, 119 aa, Artificial Sequence
  VH
QVQLVQSGAEVKKPGASVKVSCKTSGYAFTEYTMHWVRQAPGKGLEWMGGINPNTGGTTYNQKFQGRVTLTVDKSSSTAYMELSSLRSEDTVVYYCAKLLRLMYYFDYWGQGTLVTVSS

SEQ ID NO: 8 - protein, 107 aa, Artificial Sequence
  VL
DIQMTQSPSSLSASVGDRVTITCQASQDVRTAVAWYQQKPGKAPKLLIYSASYRYTGVPSRFSGSGSGTDFTFTISSLQPEDIATYYCHQHYITPWTFGGGTKVEIK

SEQ ID NO: 9 - protein, 119 aa, Artificial Sequence
  VH
QVQLVQSGAEVKKPGASVKVSCKTSGYAFTEYTMHWVRQAPGQGLEWMGGINPNTGGTTYNQKFQGRVTLTVDKSSSTAYMELSRLRSDDTVVYYCAKLLRLMYYFDYWGQGTLVTVSS

SEQ ID NO: 10 - protein, 107 aa, Artificial Sequence
  VL
DIVMTQSPDSLAVSLGERATINCKASQDVRTAVAWYQQKPGQPPKLLIYSASYRYTGVPDRFSGSGSGTDFTLTISSLQAEDVAVYYCHQHYITPWTFGGGTKVEIK

SEQ ID NO: 11 - protein, 446 aa, Artificial Sequence
  HC
QVQLVQSGAEVKKPGASVKVSCKTSGYAFTEYTMHWVRQAPGKGLEWMGGINPNTGGTTYNQKFQGRVTLTVDKSSSTAYMELSSLRSEDTVVYYCAKLLRLMYYFDYWGQGTLVTVSSASTKGPSVFPLAPCSRSTSESTAALGCLVKDYFPEPVTVSWNSGALTSGVHTFPAVLQSSGLYSLSSVVTVPSSSLGTKTYTCNVDHKPSNTKVDKRVESKYGPPCPPCPAPEFLGGPSVFLFPPKPKDTLMISRTPEVTCVVVDVSQEDPEVQFNWYVDGVEVHNAKTKPREEQFNSTYRVVSVLTVLHQDWLNGKEYKCKVSNKGLPSSIEKTISKAKGQPREPQVYTLPPSQEEMTKNQVSLTCLVKGFYPSDIAVEWESNGQPENNYKTTPPVLDSDGSFFLYSRLTVDKSRWQEGNVFSCSVMHEALHNHYTQKSLSLSLGK

SEQ ID NO: 12 - protein, 214 aa, Artificial Sequence
  LC
DIQMTQSPSSLSASVGDRVTITCQASQDVRTAVAWYQQKPGKAPKLLIYSASYRYTGVPSRFSGSGSGTDFTFTISSLQPEDIATYYCHQHYITPWTFGGGTKVEIKRTVAAPSVFIFPPSDEQLKSGTASVVCLLNNFYPREAKVQWKVDNALQSGNSQESVTEQDSKDSTYSLSSTLTLSKADYEKHKVYACEVTHQGLSSPVTKSFNRGEC

SEQ ID NO: 13 - protein, 446 aa, Artificial Sequence
  HC
QVQLVQSGAEVKKPGASVKVSCKTSGYAFTEYTMHWVRQAPGQGLEWMGGINPNTGGTTYNQKFQGRVTLTVDKSSSTAYMELSRLRSDDTVVYYCAKLLRLMYYFDYWGQGTLVTVSSASTKGPSVFPLAPCSRSTSESTAALGCLVKDYFPEPVTVSWNSGALTSGVHTFPAVLQSSGLYSLSSVVTVPSSSLGTKTYTCNVDHKPSNTKVDKRVESKYGPPCPPCPAPEFLGGPSVFLFPPKPKDTLMISRTPEVTCVVVDVSQEDPEVQFNWYVDGVEVHNAKTKPREEQFNSTYRVVSVLTVLHQDWLNGKEYKCKVSNKGLPSSIEKTISKAKGQPREPQVYTLPPSQEEMTKNQVSLTCLVKGFYPSDIAVEWESNGQPENNYKTTPPVLDSDGSFFLYSRLTVDKSRWQEGNVFSCSVMHEALHNHYTQKSLSLSLGK

SEQ ID NO: 14 - protein, 214 aa, Artificial Sequence
  LC
DIVMTQSPDSLAVSLGERATINCKASQDVRTAVAWYQQKPGQPPKLLIYSASYRYTGVPDRFSGSGSGTDFTLTISSLQAEDVAVYYCHQHYITPWTFGGGTKVEIKRTVAAPSVFIFPPSDEQLKSGTASVVCLLNNFYPREAKVQWKVDNALQSGNSQESVTEQDSKDSTYSLSSTLTLSKADYEKHKVYACEVTHQGLSSPVTKSFNRGEC